European Patent Specification EP 3 334 761 B1, published July 19, 2023. Title: Antibody-Based Molecules Selective for the {p}Ser404 Epitope of Tau and Their Uses in the Diagnosis and Treatment of Tauopathy. Applicant: New York University Sigurdsson, Einar M. The sequence listing filed with the application follows.

SEQUENCE LISTING (31 sequences)

SEQ ID NO: 1 - protein, 441 aa, Homo sapiens
  MISC_FEATURE (1)..(441): Human Tau residues
MAEPRQEFEVMEDHAGTYGLGDRKDQGGYTMHQDQEGDTDAGLKESPLQTPTEDGSEEPGSETSDAKSTPTAEDVTAPLVDEGAPGKQAAAQPHTEIPEGTTAEEAGIGDTPSLEDEAAGHVTQARMVSKSKDGTGSDDKKAKGADGKTKIATPRGAAPPGQKGQANATRIPAKTPPAPKTPPSSGEPPKSGDRSGYSSPGSPGTPGSRSRTPSLPTPPTREPKKVAVVRTPPKSPSSAKSRLQTAPVPMPDLKNVKSKIGSTENLKHQPGGGKVQIINKKLDLSNVQSKCGSKDNIKHVPGGGSVQIVYKPVDLSKVTSKCGSLGNIHHKPGGGQVEVKSEKLDFKDRVQSKIGSLDNITHVPGGGNKKIETHKLTFRENAKAKTDHGAEIVYKSPVVSGDTSPRHLSNVSSTGSIDMVDSPQLATLADEVSASLAKQGL

SEQ ID NO: 2 - protein, 15 aa, Artificial Sequence
  Glycine-Containing Linker
GGGGSGGGGSGGGGS

SEQ ID NO: 3 - protein, 18 aa, Artificial Sequence
  Linker
GSTSGSGKPGSGEGSTKG

SEQ ID NO: 4 - protein, 18 aa, Artificial Sequence
  Preferred Linker
SSGGGGSGGGGGGSSRSS

SEQ ID NO: 5 - protein, 6 aa, Artificial Sequence
  His-Tag
HHHHHH

SEQ ID NO: 6 - protein, 12 aa, Artificial Sequence
  HA-Tag
GAYPYDVPDYAS

SEQ ID NO: 7 - protein, 23 aa, Artificial Sequence
  Immunogen containing the {P}Ser404 Epitope
  MOD_RES (11)..(11): PHOSPHORYLATION (Residue is Phosphoserine)
  MOD_RES (19)..(19): PHOSPHORYLATION (Residue is Phosphoserine)
TDHGAEIVYKSPVVSGDTSPRHL

SEQ ID NO: 8 - protein, 23 aa, Artificial Sequence
  Immunogen containing the {P}Ser404 Epitope
  MOD_RES (11)..(11): PHOSPHORYLATION (Residue is Phosphoserine)
  MOD_RES (19)..(19): PHOSPHORYLATION (Residue is Phosphoserine)
TDHGAEIVYKSPVVSGDTSPRHL

SEQ ID NO: 9 - protein, 108 aa, Mus musculus
  MISC_FEATURE (1)..(108): Light Chain Variable Domain of Antibody 4E6G7
DIQMNQSPSSLSASLGDTITISCHASQNINVWLSWYQQKPGNIPKLLIFEASTLYTGVPSRFSGSGSGTGFTLTISSLQPEDIATYYCQQGQSYPWTFGGGTKLEIKR

SEQ ID NO: 10 - protein, 11 aa, Mus musculus
  MISC_FEATURE (1)..(11): CDR1 of Light Chain of Antibody 4E6G7
HASQNINVWLS

SEQ ID NO: 11 - protein, 7 aa, Mus musculus
  MISC_FEATURE (1)..(7): CDR2 of Light Chain of Antibody 4E6G7
EASTLYT

SEQ ID NO: 12 - protein, 9 aa, Mus musculus
  MISC_FEATURE (1)..(9): CDR3 of Light Chain of Antibody 4E6G7
QQGQSYPWT

SEQ ID NO: 13 - protein, 112 aa, Mus musculus
  MISC_FEATURE (1)..(112): Heavy Chain Variable Domain of Antibody 4E6G7
VQLQQSGAELVQPGASVKLSCTASGFNIKDTSMHWVRQRPEQGLEWIGRIAPANGNTKYDPKFQGKATITTDTSSNTAYLQLSSLTSEDTAVYYCSGSGNYDWGQGTTLTVS

SEQ ID NO: 14 - protein, 10 aa, Mus musculus
  MISC_FEATURE (1)..(10): CDR1 of Heavy Chain of Antibody 4E6G7
GFNIKDTSMH

SEQ ID NO: 15 - protein, 17 aa, Mus musculus
  MISC_FEATURE (1)..(17): CDR2 of Heavy Chain of Antibody 4E6G7
RIAPANGNTKYDPKFQG

SEQ ID NO: 16 - protein, 5 aa, Mus musculus
  MISC_FEATURE (1)..(5): CDR3 of Heavy Chain of Antibody 4E6G7
SGNYD

SEQ ID NO: 17 - protein, 238 aa, Artificial Sequence
  Antibody 4E6G7 scFv Fusion Protein
  MISC_FEATURE (1)..(108): Light Chain Variable Domain of Antibody 4E6G7
  MISC_FEATURE (109)..(126): Linker
  MISC_FEATURE (127)..(238): Heavy Chain Variable Domain of Antibody 4E6G7
DIQMNQSPSSLSASLGDTITISCHASQNINVWLSWYQQKPGNIPKLLIFEASTLYTGVPSRFSGSGSGTGFTLTISSLQPEDIATYYCQQGQSYPWTFGGGTKLEIKRSSGGGGSGGGGGGSSRSSVQLQQSGAELVQPGASVKLSCTASGFNIKDTSMHWVRQRPEQGLEWIGRIAPANGNTKYDPKFQGKATITTDTSSNTAYLQLSSLTSEDTAVYYCSGSGNYDWGQGTTLTVS

SEQ ID NO: 18 - protein, 28 aa, Artificial Sequence
  N-Terminal Leader Peptide
IQEEFKMKKTAIAIAVALAGFATVAQAA

SEQ ID NO: 19 - protein, 15 aa, Artificial Sequence
  C-Terminal Peptide
AKTTPPSVTSGQAGQ

SEQ ID NO: 20 - protein, 33 aa, Artificial Sequence
  C-Terminal Peptide
AKTTPPSVTSGQAGQHHHHHHGAYPYDVPDYAS

SEQ ID NO: 21 - protein, 266 aa, Artificial Sequence
  Antibody 4E6G7 scFv Fusion Protein
  MISC_FEATURE (1)..(28): N-Terminal Leader Peptide (SEQ ID NO:18)
  MISC_FEATURE (29)..(266): Antibody 4E6G7 scFv Fusion Protein (SEQ ID NO:17)
IQEEFKMKKTAIAIAVALAGFATVAQAADIQMNQSPSSLSASLGDTITISCHASQNINVWLSWYQQKPGNIPKLLIFEASTLYTGVPSRFSGSGSGTGFTLTISSLQPEDIATYYCQQGQSYPWTFGGGTKLEIKRSSGGGGSGGGGGGSSRSSVQLQQSGAELVQPGASVKLSCTASGFNIKDTSMHWVRQRPEQGLEWIGRIAPANGNTKYDPKFQGKATITTDTSSNTAYLQLSSLTSEDTAVYYCSGSGNYDWGQGTTLTVS

SEQ ID NO: 22 - protein, 253 aa, Artificial Sequence
  Antibody 4E6G7 scFv Fusion Protein
  MISC_FEATURE (1)..(238): Antibody 4E6G7 scFv Fusion Protein (SEQ ID NO:17)
  MISC_FEATURE (239)..(253): C-Terminal Peptide (SEQ ID NO:19)
DIQMNQSPSSLSASLGDTITISCHASQNINVWLSWYQQKPGNIPKLLIFEASTLYTGVPSRFSGSGSGTGFTLTISSLQPEDIATYYCQQGQSYPWTFGGGTKLEIKRSSGGGGSGGGGGGSSRSSVQLQQSGAELVQPGASVKLSCTASGFNIKDTSMHWVRQRPEQGLEWIGRIAPANGNTKYDPKFQGKATITTDTSSNTAYLQLSSLTSEDTAVYYCSGSGNYDWGQGTTLTVSAKTTPPSVTSGQAGQ

SEQ ID NO: 23 - protein, 244 aa, Artificial Sequence
  Antibody 4E6G7 scFv Fusion Protein
  MISC_FEATURE (1)..(238): Antibody 4E6G7 scFv Fusion Protein (SEQ ID NO:17)
  MISC_FEATURE (239)..(244): C-Terminal Peptide (SEQ ID NO:5)
DIQMNQSPSSLSASLGDTITISCHASQNINVWLSWYQQKPGNIPKLLIFEASTLYTGVPSRFSGSGSGTGFTLTISSLQPEDIATYYCQQGQSYPWTFGGGTKLEIKRSSGGGGSGGGGGGSSRSSVQLQQSGAELVQPGASVKLSCTASGFNIKDTSMHWVRQRPEQGLEWIGRIAPANGNTKYDPKFQGKATITTDTSSNTAYLQLSSLTSEDTAVYYCSGSGNYDWGQGTTLTVSHHHHHH

SEQ ID NO: 24 - protein, 250 aa, Artificial Sequence
  Antibody 4E6G7 scFv Fusion Protein
  MISC_FEATURE (1)..(238): Antibody 4E6G7 scFv Fusion Protein (SEQ ID NO:17)
  MISC_FEATURE (239)..(250): C-Terminal Peptide (SEQ ID NO:6)
DIQMNQSPSSLSASLGDTITISCHASQNINVWLSWYQQKPGNIPKLLIFEASTLYTGVPSRFSGSGSGTGFTLTISSLQPEDIATYYCQQGQSYPWTFGGGTKLEIKRSSGGGGSGGGGGGSSRSSVQLQQSGAELVQPGASVKLSCTASGFNIKDTSMHWVRQRPEQGLEWIGRIAPANGNTKYDPKFQGKATITTDTSSNTAYLQLSSLTSEDTAVYYCSGSGNYDWGQGTTLTVSGAYPYDVPDYAS

SEQ ID NO: 25 - protein, 271 aa, Artificial Sequence
  Antibody 4E6G7 scFv Fusion Protein
  MISC_FEATURE (1)..(238): Antibody 4E6G7 scFv Fusion Protein (SEQ ID NO:17)
  MISC_FEATURE (239)..(271): C-Terminal Peptide (SEQ ID NO:20)
DIQMNQSPSSLSASLGDTITISCHASQNINVWLSWYQQKPGNIPKLLIFEASTLYTGVPSRFSGSGSGTGFTLTISSLQPEDIATYYCQQGQSYPWTFGGGTKLEIKRSSGGGGSGGGGGGSSRSSVQLQQSGAELVQPGASVKLSCTASGFNIKDTSMHWVRQRPEQGLEWIGRIAPANGNTKYDPKFQGKATITTDTSSNTAYLQLSSLTSEDTAVYYCSGSGNYDWGQGTTLTVSAKTTPPSVTSGQAGQHHHHHHGAYPYDVPDYAS

SEQ ID NO: 26 - protein, 281 aa, Artificial Sequence
  Antibody 4E6G7 scFv Fusion Protein
  MISC_FEATURE (1)..(28): N-Terminal Leader Peptide (SEQ ID NO:18)
  MISC_FEATURE (29)..(266): Antibody 4E6G7 scFv Fusion Protein (SEQ ID NO:17)
  MISC_FEATURE (267)..(281): C-Terminal Peptide (SEQ ID NO:5)
IQEEFKMKKTAIAIAVALAGFATVAQAADIQMNQSPSSLSASLGDTITISCHASQNINVWLSWYQQKPGNIPKLLIFEASTLYTGVPSRFSGSGSGTGFTLTISSLQPEDIATYYCQQGQSYPWTFGGGTKLEIKRSSGGGGSGGGGGGSSRSSVQLQQSGAELVQPGASVKLSCTASGFNIKDTSMHWVRQRPEQGLEWIGRIAPANGNTKYDPKFQGKATITTDTSSNTAYLQLSSLTSEDTAVYYCSGSGNYDWGQGTTLTVSAKTTPPSVTSGQAGQ

SEQ ID NO: 27 - protein, 272 aa, Artificial Sequence
  Antibody 4E6G7 scFv Fusion Protein
  MISC_FEATURE (1)..(28): N-Terminal Leader Peptide (SEQ ID NO:18)
  MISC_FEATURE (29)..(266): Antibody 4E6G7 scFv Fusion Protein (SEQ ID NO:17)
  MISC_FEATURE (267)..(272): C-Terminal Peptide (SEQ ID NO:18)
IQEEFKMKKTAIAIAVALAGFATVAQAADIQMNQSPSSLSASLGDTITISCHASQNINVWLSWYQQKPGNIPKLLIFEASTLYTGVPSRFSGSGSGTGFTLTISSLQPEDIATYYCQQGQSYPWTFGGGTKLEIKRSSGGGGSGGGGGGSSRSSVQLQQSGAELVQPGASVKLSCTASGFNIKDTSMHWVRQRPEQGLEWIGRIAPANGNTKYDPKFQGKATITTDTSSNTAYLQLSSLTSEDTAVYYCSGSGNYDWGQGTTLTVSHHHHHH

SEQ ID NO: 28 - protein, 278 aa, Artificial Sequence
  Antibody 4E6G7 scFv Fusion Protein
  MISC_FEATURE (1)..(28): N-Terminal Leader Peptide (SEQ ID NO:18)
  MISC_FEATURE (29)..(266): Antibody 4E6G7 scFv Fusion Protein (SEQ ID NO:17)
  MISC_FEATURE (267)..(278): C-Terminal Peptide (SEQ ID NO:6)
IQEEFKMKKTAIAIAVALAGFATVAQAADIQMNQSPSSLSASLGDTITISCHASQNINVWLSWYQQKPGNIPKLLIFEASTLYTGVPSRFSGSGSGTGFTLTISSLQPEDIATYYCQQGQSYPWTFGGGTKLEIKRSSGGGGSGGGGGGSSRSSVQLQQSGAELVQPGASVKLSCTASGFNIKDTSMHWVRQRPEQGLEWIGRIAPANGNTKYDPKFQGKATITTDTSSNTAYLQLSSLTSEDTAVYYCSGSGNYDWGQGTTLTVSGAYPYDVPDYAS

SEQ ID NO: 29 - protein, 299 aa, Artificial Sequence
  Antibody 4E6G7 scFv Fusion Protein
  MISC_FEATURE (1)..(28): N-Terminal Leader Peptide (SEQ ID NO:18)
  MISC_FEATURE (29)..(266): Antibody 4E6G7 scFv Fusion Protein (SEQ ID NO:17)
  MISC_FEATURE (267)..(299): C-Terminal Peptide (SEQ ID NO:20)
IQEEFKMKKTAIAIAVALAGFATVAQAADIQMNQSPSSLSASLGDTITISCHASQNINVWLSWYQQKPGNIPKLLIFEASTLYTGVPSRFSGSGSGTGFTLTISSLQPEDIATYYCQQGQSYPWTFGGGTKLEIKRSSGGGGSGGGGGGSSRSSVQLQQSGAELVQPGASVKLSCTASGFNIKDTSMHWVRQRPEQGLEWIGRIAPANGNTKYDPKFQGKATITTDTSSNTAYLQLSSLTSEDTAVYYCSGSGNYDWGQGTTLTVSAKTTPPSVTSGQAGQHHHHHHGAYPYDVPDYAS

SEQ ID NO: 30 - protein, 30 aa, Artificial Sequence
  Tau 379-408 ({p}Ser396/{p}Ser404)
  MOD_RES (18)..(18): PHOSPHORYLATION (residue is phosphoserine)
  MOD_RES (26)..(26): PHOSPHORYLATION (residue is phosphoserine)
RENAKAKTDHGAEIVYKSPVVSGDTSPRHL

SEQ ID NO: 31 - protein, 30 aa, Homo sapiens; identical to SEQ ID NO: 30
  MISC_FEATURE (1)..(30): Tau 379-408